European Patent Specification EP 3 639 838 B1, published November 8, 2023. Title: MILK-BASED PROTEIN HYDROLYSATES. Applicant: NESTEC S.A. The sequence listing filed with the application follows.

SEQUENCE LISTING (1 sequence)

SEQ ID NO: 1 - protein, 225 aa, Kutzneria albida
  SOURCE 1..225: /mol_type="protein" /organism="Kutzneria albida"
IVGGTKASTSTYPFVVFLTDSTGFQFCGGTLVKPNKVVTAAHCTVGESAANIRVVAGRDDKQSTAGTVSKVSKIWIHPSYQDATKGSDVSVLTLSTSLTQFTPLPLAATTDTALYKEGTAATILGWGDTTEGGSASRYLLKATVPLTSDATCKKAYGEYSSTAMVCAGYPQGGTDTCQGDSGGPLVAGNKLIGITSWGQGCAEAGYPGVYTRVATYSSLITQQLG